European Patent Application EP 4 159 753 A1, published April 5, 2023. Title: T CELL RECEPTORS RECOGNIZING MHC CLASS II-RESTRICTED MAGE-A3. Applicant: THE UNITED STATES OF AMERICA, AS REPRESENTED BY THE SECRETARY, DEPARTMENT OF HEALTH AND HUMAN SERVICES. Application EP - not yet assigned. The sequence listing filed with the application follows.

SEQUENCE LISTING (71 sequences)

SEQ ID NO: 1 - protein, 314 aa, Homo sapiens
MPLEQRSQHCKPEEGLEARGEALGLVGAQAPATEEQEAASSSSTLVEVTLGEVPAAESPDPPQSPQGASSLPTTMNYPLWSQSYEDSSNQEEEGPSTFPDLESEFQAALSRKVAELVHFLLLKYRAREPVTKAEMLGSVVGNWQYFFPVIFSKASSSLQLVFGIELMEVDPIGHLYIFATCLGLSYDGLLGDNQIMPKAGLLIIVLAIIAREGDCAPEEKIWEELSVLEVFEGREDSILGDPKKLLTQHFVQENYLEYRQVPGSDPACYEFLWGPRALVETSYVKVLHHMVKISGGPHISYPPLHEWVLREGEE

SEQ ID NO: 2 - protein, 16 aa, Homo sapiens
KKLLTQHFVQENYLEY

SEQ ID NO: 3 - protein, 7 aa, Homo sapiens
TSESDYY

SEQ ID NO: 4 - protein, 7 aa, Homo sapiens
QEAYKQQ

SEQ ID NO: 5 - protein, 11 aa, Homo sapiens
ALRSSGTYKYI

SEQ ID NO: 6 - protein, 5 aa, Homo sapiens
SGHTA

SEQ ID NO: 7 - protein, 6 aa, Homo sapiens
FQGNSA

SEQ ID NO: 8 - protein, 15 aa, Homo sapiens
ASIRTGPFFSGNTIY

SEQ ID NO: 9 - protein, 134 aa, Homo sapiens
MACPGFLWALVISTCLEFSMAQTVTQSQPEMSVQEAETVTLSCTYDTSESDYYLFWYKQPPSRQMILVIRQEAYKQQNATENRFSVNFQKAAKSFSLKISDSQLGDAAMYFCALRSSGTYKYIFGTGTRLKVLA

SEQ ID NO: 10 - protein, 137 aa, Homo sapiens
MGTRLLFWVAFCLLGADHTGAGVSQSPSNKVTEKGKDVELRCDPISGHTALYWYRQSLGQGLEFLIYFQGNSAPDKSGLPSDRFSAERTGGSVSTLTIQRTQQEDSAVYLCASIRTGPFFSGNTIYFGEGSWLTVVE

SEQ ID NO: 11 - protein, 275 aa, Homo sapiens
MACPGFLWALVISTCLEFSMAQTVTQSQPEMSVQEAETVTLSCTYDTSESDYYLFWYKQPPSRQMILVIRQEAYKQQNATENRFSVNFQKAAKSFSLKISDSQLGDAAMYFCALRSSGTYKYIFGTGTRLKVLANIQNPDPAVYQLRDSKSSDKSVCLFTDFDSQTNVSQSKDSDVYITDKTVLDMRSMDFKSNSAVAWSNKSDFACANAFNNSIIPEDTFFPSPESSCDVKLVEKSFETDTNLNFQNLSVIGFRILLLKVAGFNLLMTLRLWSS

SEQ ID NO: 12 - protein, 313 aa, Homo sapiens
MGTRLLFWVAFCLLGADHTGAGVSQSPSNKVTEKGKDVELRCDPISGHTALYWYRQSLGQGLEFLIYFQGNSAPDKSGLPSDRFSAERTGGSVSTLTIQRTQQEDSAVYLCASIRTGPFFSGNTIYFGEGSWLTVVEDLNKVFPPEVAVFEPSEAEISHTQKATLVCLATGFFPDHVELSWWVNGKEVHSGVSTDPQPLKEQPALNDSRYCLSSRLRVSATFWQNPRNHFRCQVQFYGLSENDEWTQDRAKPVTQIVSAEAWGRADCGFTSVSYQQGVLSATILYEILLGKATLYAVLVSALVLMAMVKRKDF

SEQ ID NO: 13 - protein, 7 aa, Homo sapiens
TSESDYY

SEQ ID NO: 14 - protein, 7 aa, Homo sapiens
QEAYKQQ

SEQ ID NO: 15 - protein, 17 aa, Homo sapiens
AYTVPSNAGGTSYGKLT

SEQ ID NO: 16 - protein, 5 aa, Homo sapiens
SNHLY

SEQ ID NO: 17 - protein, 6 aa, Homo sapiens
FYNNEI

SEQ ID NO: 18 - protein, 12 aa, Homo sapiens
ASSERGQGYGYT

SEQ ID NO: 19 - protein, 140 aa, Homo sapiens
MACPGFLWALVISTCLEFSMAQTVTQSQPEMSVQEAETVTLSCTYDTSESDYYLFWYKQPPSRQMILVIRQEAYKQQNATENRFSVNFQKAAKSFSLKISDSQLGDAAMYFCAYTVPSNAGGTSYGKLTFGQGTILTVHP

SEQ ID NO: 20 - protein, 134 aa, Homo sapiens
MDTWLVCWAIFSLLKAGLTEPEVTQTPSHQVTQMGQEVILRCVPISNHLYFYWYRQILGQKVEFLVSFYNNEISEKSEIFDDQFSVERPDGSNFTLKIRSTKLEDSAMYFCASSERGQGYGYTFGSGTRLTVVE

SEQ ID NO: 21 - protein, 281 aa, Homo sapiens [sequence omitted]

SEQ ID NO: 22 - protein, 310 aa, Homo sapiens
MDTWLVCWAIFSLLKAGLTEPEVTQTPSHQVTQMGQEVILRCVPISNHLYFYWYRQILGQKVEFLVSFYNNEISEKSEIFDDQFSVERPDGSNFTLKIRSTKLEDSAMYFCASSERGQGYGYTFGSGTRLTVVEDLNKVFPPEVAVFEPSEAEISHTQKATLVCLATGFFPDHVELSWWVNGKEVHSGVSTDPQPLKEQPALNDSRYCLSSRLRVSATFWQNPRNHFRCQVQFYGLSENDEWTQDRAKPVTQIVSAEAWGRADCGFTSVSYQQGVLSATILYEILLGKATLYAVLVSALVLMAMVKRKDF

SEQ ID NO: 23 - protein, 141 aa, Homo sapiens
NIQNPDPAVYQLRDSKSSDKSVCLFTDFDSQTNVSQSKDSDVYITDKTVLDMRSMDFKSNSAVAWSNKSDFACANAFNNSIIPEDTFFPSPESSCDVKLVEKSFETDTNLNFQNLSVIGFRILLLKVAGFNLLMTLRLWSS

SEQ ID NO: 24 - protein, 176 aa, Homo sapiens
DLNKVFPPEVAVFEPSEAEISHTQKATLVCLATGFFPDHVELSWWVNGKEVHSGVSTDPQPLKEQPALNDSRYCLSSRLRVSATFWQNPRNHFRCQVQFYGLSENDEWTQDRAKPVTQIVSAEAWGRADCGFTSVSYQQGVLSATILYEILLGKATLYAVLVSALVLMAMVKRKDF

SEQ ID NO: 25 - protein, 137 aa, Mus musculus
NIQNPEPAVYQLKDPRSQDSTLCLFTDFDSQINVPKTMESGTFITDKTVLDMKAMDSKSNGAIAWSNQTSFTCQDIFKETNATYPSSDVPCDATLTEKSFETDMNLNFQNLSVMGLRILLLKVAGFNLLMTLRLWSS

SEQ ID NO: 26 - protein, 172 aa, Mus musculus
DLRNVTPPKVSLFEPSKAEIANKQKATLVCLARGFFPDHVELSWWVNGKEVHSGVSTDPQAYKESNYSYCLSSRLRVSATFWHNPRNHFRCQVQFHGLSEEDKWPEGSPKPVTQNISAEAWGRADCGITSASYHQGVLSATILYEILLGKATLYAVLVSGLVLMAMVKRKNS

SEQ ID NO: 27 - protein, 271 aa, Artificial Sequence
  Synthetic
MACPGFLWALVISTCLEFSMAQTVTQSQPEMSVQEAETVTLSCTYDTSESDYYLFWYKQPPSRQMILVIRQEAYKQQNATENRFSVNFQKAAKSFSLKISDSQLGDAAMYFCALRSSGTYKYIFGTGTRLKVLANIQNPEPAVYQLKDPRSQDSTLCLFTDFDSQINVPKTMESGTFITDKTVLDMKAMDSKSNGAIAWSNQTSFTCQDIFKETNATYPSSDVPCDATLTEKSFETDMNLNFQNLSVMGLRILLLKVAGFNLLMTLRLWSS

SEQ ID NO: 28 - protein, 309 aa, Artificial Sequence
  Synthetic
MGTRLLFWVAFCLLGADHTGAGVSQSPSNKVTEKGKDVELRCDPISGHTALYWYRQSLGQGLEFLIYFQGNSAPDKSGLPSDRFSAERTGGSVSTLTIQRTQQEDSAVYLCASIRTGPFFSGNTIYFGEGSWLTVVEDLRNVTPPKVSLFEPSKAEIANKQKATLVCLARGFFPDHVELSWWVNGKEVHSGVSTDPQAYKESNYSYCLSSRLRVSATFWHNPRNHFRCQVQFHGLSEEDKWPEGSPKPVTQNISAEAWGRADCGITSASYHQGVLSATILYEILLGKATLYAVLVSGLVLMAMVKRKNS

SEQ ID NO: 29 - protein, 11 aa, Artificial Sequence
  Synthetic
  site (4)..(5): X at 4  and 5 is Ser, Ala, Leu, Ile, Val, or Met
  site (6)..(6): X at 6 is Gly, Ala, Leu, Ile, Val, or Met
  site (7)..(7): X at 7 is Thr, Ala, Leu, Ile, Val, or Met
  site (7)..(7): X at 7 is Thr, Ala, Leu, Ile, Val, or Met
ALRXXXXYKYI

SEQ ID NO: 30 - protein, 15 aa, Artificial Sequence
  Synthetic
  site (4)..(4): X at 4 is Arg, Ala, Leu, Ile, Val, or Met
  site (5)..(5): X at 5 is Thr, Ala, Leu, Ile, Val, or Met
  site (6)..(6): X at 6 is Gly, Ala, Leu, Ile, Val, or Met
  site (7)..(7): X at 7 is Pro, Ala, Leu, Ile, Val, or Met
ASIXXXXFFSGNTIY

SEQ ID NO: 31 - protein, 134 aa, Artificial Sequence
  Synthetic
  site (116)..(117)
  site (116)..(117)
  site (118)..(118)
  site (119)..(119)
MACPGFLWALVISTCLEFSMAQTVTQSQPEMSVQEAETVTLSCTYDTSESDYYLFWYKQPPSRQMILVIRQEAYKQQNATENRFSVNFQKAAKSFSLKISDSQLGDAAMYFCALRXXXXYKYIFGTGTRLKVLA

SEQ ID NO: 32 - protein, 137 aa, Artificial Sequence
  Synthetic
  site (115)..(115): X at 115 is Arg, Ala, Leu, Ile, Val, or Met
  site (116)..(116): X at 116 is Thr, Ala, Leu, Ile, Val, or Met
  site (117)..(117): X at 117 is Gly, Ala, Leu, Ile, Val, or Met
  site (118)..(118): X at 118 is Pro, Ala, Leu, Ile, Val, or Met
MGTRLLFWVAFCLLGADHTGAGVSQSPSNKVTEKGKDVELRCDPISGHTALYWYRQSLGQGLEFLIYFQGNSAPDKSGLPSDRFSAERTGGSVSTLTIQRTQQEDSAVYLCASIXXXXFFSGNTIYFGEGSWLTVVE

SEQ ID NO: 33 - protein, 275 aa, Artificial Sequence
  Synthetic
  site (116)..(117): X at 116  and 117 is Ser, Ala, Leu, Ile, Val, or Met
  site (118)..(118): X at 118 is Gly, Ala, Leu, Ile, Val, or Met
  site (119)..(119): X at 119 is Thr, Ala, Leu, Ile, Val, or Met
MACPGFLWALVISTCLEFSMAQTVTQSQPEMSVQEAETVTLSCTYDTSESDYYLFWYKQPPSRQMILVIRQEAYKQQNATENRFSVNFQKAAKSFSLKISDSQLGDAAMYFCALRXXXXYKYIFGTGTRLKVLANIQNPDPAVYQLRDSKSSDKSVCLFTDFDSQTNVSQSKDSDVYITDKTVLDMRSMDFKSNSAVAWSNKSDFACANAFNNSIIPEDTFFPSPESSCDVKLVEKSFETDTNLNFQNLSVIGFRILLLKVAGFNLLMTLRLWSS

SEQ ID NO: 34 - protein, 313 aa, Artificial Sequence
  Synthetic
  site (115)..(115): X at 115 is Arg, Ala, Leu, Ile, Val, or Met
  site (116)..(116): X at 116 is Thr, Ala, Leu, Ile, Val, or Met
  site (117)..(117): X at 117 is Gly, Ala, Leu, Ile, Val, or Met
  site (118)..(118): X at 118 is Pro, Ala, Leu, Ile, Val, or Met
MGTRLLFWVAFCLLGADHTGAGVSQSPSNKVTEKGKDVELRCDPISGHTALYWYRQSLGQGLEFLIYFQGNSAPDKSGLPSDRFSAERTGGSVSTLTIQRTQQEDSAVYLCASIXXXXFFSGNTIYFGEGSWLTVVEDLNKVFPPEVAVFEPSEAEISHTQKATLVCLATGFFPDHVELSWWVNGKEVHSGVSTDPQPLKEQPALNDSRYCLSSRLRVSATFWQNPRNHFRCQVQFYGLSENDEWTQDRAKPVTQIVSAEAWGRADCGFTSVSYQQGVLSATILYEILLGKATLYAVLVSALVLMAMVKRKDF

SEQ ID NO: 35 - protein, 141 aa, Homo sapiens; identical to SEQ ID NO: 23

SEQ ID NO: 36 - protein, 176 aa, Homo sapiens; identical to SEQ ID NO: 24

SEQ ID NO: 37 - DNA, 828 bp, Homo sapiens
atggcatgccctggcttcctgtgggcacttgtgatctccacctgtcttgaatttagcatggctcagacagtcactcagtctcaaccagagatgtctgtgcaggaggcagagaccgtgaccctgagctgcacatatgacaccagtgagagtgattattatttattctggtacaagcagcctcccagcaggcagatgattctcgttattcgccaagaagcttataagcaacagaatgcaacagagaatcgtttctctgtgaacttccagaaagcagccaaatccttcagtctcaagatctcagactcacagctgggggatgccgcgatgtatttctgtgctctccggagctcaggaacctacaaatacatctttggaacaggcaccaggctgaaggttttagcaaatatccagaaccctgaccctgccgtgtaccagctgagagactctaaatccagtgacaagtctgtctgcctattcaccgattttgattctcaaacaaatgtgtcacaaagtaaggattctgatgtgtatatcacagacaaaactgtgctagacatgaggtctatggacttcaagagcaacagtgctgtggcctggagcaacaaatctgactttgcatgtgcaaacgccttcaacaacagcattattccagaagacaccttcttccccagcccagaaagttcctgtgatgtcaagctggtcgagaaaagctttgaaacagatacgaacctaaactttcaaaacctgtcagtgattgggttccgaatcctcctcctgaaagtggccgggtttaatctgctcatgacgctgcggctgtggtccagctga

SEQ ID NO: 38 - DNA, 942 bp, Homo sapiens
atgggcaccaggctcctcttctgggtggccttctgtctcctgggggcagatcacacaggagctggagtctcccagtcccccagtaacaaggtcacagagaagggaaaggatgtagagctcaggtgtgatccaatttcaggtcatactgccctttactggtaccgacagagcctggggcagggcctggagtttttaatttacttccaaggcaacagtgcaccagacaaatcagggctgcccagtgatcgcttctctgcagagaggactgggggatccgtctccactctgacgatccagcgcacacagcaggaggactcggccgtgtatctctgtgccagcatccggacagggccttttttctctggaaacaccatatattttggagagggaagttggctcactgttgtagaggacctgaacaaggtgttcccacccgaggtcgctgtgtttgagccatcagaagcagagatctcccacacccaaaaggccacactggtgtgcctggccacaggcttcttccctgaccacgtggagctgagctggtgggtgaatgggaaggaggtgcacagtggggtcagcacggacccgcagcccctcaaggagcagcccgccctcaatgactccagatactgcctgagcagccgcctgagggtctcggccaccttctggcagaacccccgcaaccacttccgctgtcaagtccagttctacgggctctcggagaatgacgagtggacccaggatagggccaaacccgtcacccagatcgtcagcgccgaggcctggggtagagcagactgtggctttacctcggtgtcctaccagcaaggggtcctgtctgccaccatcctctatgagatcctgctagggaaggccaccctgtatgctgtgctggtcagcgcccttgtgttgatggccatggtcaagagaaaggatttctga

SEQ ID NO: 39 - DNA, 846 bp, Homo sapiens
atggcatgccctggcttcctgtgggcacttgtgatctccacctgtcttgaatttagcatggctcagacagtcactcagtctcaaccagagatgtctgtgcaggaggcagagaccgtgaccctgagctgcacatatgacaccagtgagagtgattattatttattctggtacaagcagcctcccagcaggcagatgattctcgttattcgccaagaagcttataagcaacagaatgcaacagagaatcgtttctctgtgaacttccagaaagcagccaaatccttcagtctcaagatctcagactcacagctgggggatgccgcgatgtatttctgtgcttacacggttccctctaatgctggtggtactagctatggaaagctgacatttggacaagggaccatcttgactgtccatccaaatatccagaaccctgaccctgccgtgtaccagctgagagactctaaatccagtgacaagtctgtctgcctattcaccgattttgattctcaaacaaatgtgtcacaaagtaaggattctgatgtgtatatcacagacaaaactgtgctagacatgaggtctatggacttcaagagcaacagtgctgtggcctggagcaacaaatctgactttgcatgtgcaaacgccttcaacaacagcattattccagaagacaccttcttccccagcccagaaagttcctgtgatgtcaagctggtcgagaaaagctttgaaacagatacgaacctaaactttcaaaacctgtcagtgattgggttccgaatcctcctcctgaaagtggccgggtttaatctgctcatgacgctgcggctgtggtccagctga

SEQ ID NO: 40 - DNA, 933 bp, Homo sapiens
atggatacctggctcgtatgctgggcaatttttagtctcttgaaagcaggactcacagaacctgaagtcacccagactcccagccatcaggtcacacagatgggacaggaagtgatcttgcgctgtgtccccatctctaatcacttatacttctattggtacagacaaatcttggggcagaaagtcgagtttctggtttccttttataataatgaaatctcagagaagtctgaaatattcgatgatcaattctcagttgaaaggcctgatggatcaaatttcactctgaagatccggtccacaaagctggaggactcagccatgtacttctgtgccagcagtgaaaggggacagggttatggctacaccttcggttcggggaccaggttaaccgttgtagaggacctgaacaaggtgttcccacccgaggtcgctgtgtttgagccatcagaagcagagatctcccacacccaaaaggccacactggtgtgcctggccacaggcttcttccccgaccacgtggagctgagctggtgggtgaatgggaaggaggtgcacagtggggtcagcacagacccgcagcccctcaaggagcagcccgccctcaatgactccagatactgcctgagcagccgcctgagggtctcggccaccttctggcagaacccccgcaaccacttccgctgtcaagtccagttctacgggctctcggagaatgacgagtggacccaggatagggccaaacccgtcacccagatcgtcagcgccgaggcctggggtagagcagactgtggctttacctcggtgtcctaccagcaaggggtcctgtctgccaccatcctctatgagatcctgctagggaaggccaccctgtatgctgtgctggtcagcgcccttgtgttgatggccatggtcaagagaaaggatttctga

SEQ ID NO: 41 - DNA, 816 bp, Artificial Sequence
  Synthetic
atggcatgccctggcttcctgtgggcacttgtgatctccacctgtcttgaatttagcatggctcagacagtcactcagtctcaaccagagatgtctgtgcaggaggcagagaccgtgaccctgagctgcacatatgacaccagtgagagtgattattatttattctggtacaagcagcctcccagcaggcagatgattctcgttattcgccaagaagcttataagcaacagaatgcaacagagaatcgtttctctgtgaacttccagaaagcagccaaatccttcagtctcaagatctcagactcacagctgggggatgccgcgatgtatttctgtgctctccggagctcaggaacctacaaatacatctttggaacaggcaccaggctgaaggttttagcaaatatccagaaccctgaacctgctgtgtaccagttaaaagatcctcggtctcaggacagcaccctctgcctgttcaccgactttgactcccaaatcaatgtgccgaaaaccatggaatctggaacgttcatcactgacaaaactgtgctggacatgaaagctatggattccaagagcaatggggccattgcctggagcaaccagacaagcttcacctgccaagatatcttcaaagagaccaacgccacctaccccagttcagacgttccctgtgatgccacgttgactgagaaaagctttgaaacagatatgaacctaaactttcaaaacctgtcagttatgggactccgaatcctcctgctgaaagtagccggatttaacctgctcatgacgctgaggctgtggtccagttga

SEQ ID NO: 42 - DNA, 930 bp, Artificial Sequence
  Synthetic
atgggcaccaggctcctcttctgggtggccttctgtctcctgggggcagatcacacaggagctggagtctcccagtcccccagtaacaaggtcacagagaagggaaaggatgtagagctcaggtgtgatccaatttcaggtcatactgccctttactggtaccgacagagcctggggcagggcctggagtttttaatttacttccaaggcaacagtgcaccagacaaatcagggctgcccagtgatcgcttctctgcagagaggactgggggatccgtctccactctgacgatccagcgcacacagcaggaggactcggccgtgtatctctgtgccagcatccggacagggccttttttctctggaaacaccatatattttggagagggaagttggctcactgttgtagaggacctgagaaacgtgaccccacccaaggtctccttgtttgagccatcaaaagcagagattgcaaacaaacaaaaggctaccctcgtgtgcttggccaggggcttcttccctgaccacgtggagctgagctggtgggtgaatggcaaggaggtccacagtggggtcagcacggaccctcaggcctacaaggagagcaattatagctactgcctgagcagccgcctgagggtctctgctaccttctggcacaatcctcgaaaccacttccgctgccaagtgcagttccatgggctttcagaggaggacaagtggccagagggctcacccaaacctgtcacacagaacatcagtgcagaggcctggggccgagcagactgtggaatcacttcagcatcctatcatcagggggttctgtctgcaaccatcctctatgagatcctactggggaaggccaccctatatgctgtgctggtcagtggcctggtgctgatggctatggtcaaaagaaagaactcatga

SEQ ID NO: 43 - DNA, 828 bp, Artificial Sequence
  Synthetic
  misc_feature (346)..(348): nnn at 346-348 is AGC, GCC, or any codon that encodes Ser, Ala, Leu, Ile, Val, or Met
  misc_feature (349)..(351): nnn at 349-351 is TCA, GCC, or any codon that encodes Ser, Ala, Leu, Ile, Val, or Met
  misc_feature (352)..(354): 352-354 is GGA, GCC, or any codon that encodes Gly, Ala, Leu, Ile, Val, or Met
  misc_feature (355)..(357): nnn at misc feature: nnn at 355-357 is ACC, GCC, or any codon that encodes Thr, Ala, Leu, Ile, Val, or Met
atggcatgccctggcttcctgtgggcacttgtgatctccacctgtcttgaatttagcatggctcagacagtcactcagtctcaaccagagatgtctgtgcaggaggcagagaccgtgaccctgagctgcacatatgacaccagtgagagtgattattatttattctggtacaagcagcctcccagcaggcagatgattctcgttattcgccaagaagcttataagcaacagaatgcaacagagaatcgtttctctgtgaacttccagaaagcagccaaatccttcagtctcaagatctcagactcacagctgggggatgccgcgatgtatttctgtgctctccggnnnnnnnnnnnntacaaatacatctttggaacaggcaccaggctgaaggttttagcaaatatccagaaccctgaccctgccgtgtaccagctgagagactctaaatccagtgacaagtctgtctgcctattcaccgattttgattctcaaacaaatgtgtcacaaagtaaggattctgatgtgtatatcacagacaaaactgtgctagacatgaggtctatggacttcaagagcaacagtgctgtggcctggagcaacaaatctgactttgcatgtgcaaacgccttcaacaacagcattattccagaagacaccttcttccccagcccagaaagttcctgtgatgtcaagctggtcgagaaaagctttgaaacagatacgaacctaaactttcaaaacctgtcagtgattgggttccgaatcctcctcctgaaagtggccgggtttaatctgctcatgacgctgcggctgtggtccagctga

SEQ ID NO: 44 - DNA, 942 bp, Artificial Sequence
  Synthetic
  misc_feature (343)..(345): NNN at 343-345 is CGG, GCC, or any codon that encodes Arg, Ala, Leu, Ile, Val, or Met
  misc_feature (346)..(348): NNN at 346-348 is ACA, GCC, or any codon that encodes Thr, Ala, Leu, Ile, Val, or Met
  misc_feature (349)..(351): NNN at 349-351 is GGG, GCC, or any codon that encodes Gly, Ala, Leu, Ile, Val, or Met
  misc_feature (352)..(354): NNN at 352-354 is CCT, GCC, or any codon that encodes Pro, Ala, Leu, Ile, Val, or Met
atgggcaccaggctcctcttctgggtggccttctgtctcctgggggcagatcacacaggagctggagtctcccagtcccccagtaacaaggtcacagagaagggaaaggatgtagagctcaggtgtgatccaatttcaggtcatactgccctttactggtaccgacagagcctggggcagggcctggagtttttaatttacttccaaggcaacagtgcaccagacaaatcagggctgcccagtgatcgcttctctgcagagaggactgggggatccgtctccactctgacgatccagcgcacacagcaggaggactcggccgtgtatctctgtgccagcatcnnnnnnnnnnnntttttctctggaaacaccatatattttggagagggaagttggctcactgttgtagaggacctgaacaaggtgttcccacccgaggtcgctgtgtttgagccatcagaagcagagatctcccacacccaaaaggccacactggtgtgcctggccacaggcttcttccctgaccacgtggagctgagctggtgggtgaatgggaaggaggtgcacagtggggtcagcacggacccgcagcccctcaaggagcagcccgccctcaatgactccagatactgcctgagcagccgcctgagggtctcggccaccttctggcagaacccccgcaaccacttccgctgtcaagtccagttctacgggctctcggagaatgacgagtggacccaggatagggccaaacccgtcacccagatcgtcagcgccgaggcctggggtagagcagactgtggctttacctcggtgtcctaccagcaaggggtcctgtctgccaccatcctctatgagatcctgctagggaaggccaccctgtatgctgtgctggtcagcgcccttgtgttgatggccatggtcaagagaaaggatttctga

SEQ ID NO: 45 - protein, 314 aa, Homo sapiens
MPLEQRSQHCKPEEGLEARGEALGLVGAQAPATEEQEAASSSSTLVEVTLGEVPAAESPDPPQSPQGASSLPTTMNYPLWSQSYEDSSNQEEEGPSTFPDLESEFQAALSRKVAKLVHFLLLKYRAREPVTKAEMLGSVVGNWQYFFPVIFSKASDSLQLVFGIELMEVDPIGHVYIFATCLGLSYDGLLGDNQIMPKTGFLIIILAIIAKEGDCAPEEKIWEELSVLEVFEGREDSIFGDPKKLLTQYFVQENYLEYRQVPGSDPACYEFLWGPRALIETSYVKVLHHMVKISGGPRISYPLLHEWALREGEE

SEQ ID NO: 46 - protein, 16 aa, Homo sapiens
KKLLTQYFVQENYLEY

SEQ ID NO: 47 - protein, 14 aa, Artificial Sequence
  Synthetic
KKLLTQHFVQENYL

SEQ ID NO: 48 - protein, 13 aa, Artificial Sequence
  Synthetic
KKLLTQHFVQENY

SEQ ID NO: 49 - protein, 12 aa, Artificial Sequence
  Synthetic
KKLLTQHFVQEN

SEQ ID NO: 50 - protein, 11 aa, Artificial Sequence
  Synthetic
KKLLTQHFVQE

SEQ ID NO: 51 - protein, 14 aa, Artificial Sequence
  Synthetic
LLTQHFVQENYLEY

SEQ ID NO: 52 - protein, 13 aa, Artificial Sequence
  Synthetic
LTQHFVQENYLEY

SEQ ID NO: 53 - protein, 12 aa, Artificial Sequence
  Synthetic
TQHFVQENYLEY

SEQ ID NO: 54 - protein, 11 aa, Artificial Sequence
  Synthetic
QHFVQENYLEY

SEQ ID NO: 55 - protein, 10 aa, Artificial Sequence
  Synthetic
HFVQENYLEY

SEQ ID NO: 56 - protein, 11 aa, Artificial Sequence
  Synthetic
QYFVQENYLEY

SEQ ID NO: 57 - protein, 11 aa, Artificial Sequence
  Synthetic
QDLVQENYLEY

SEQ ID NO: 58 - protein, 11 aa, Artificial Sequence
  Synthetic
QDWVQENYLEY

SEQ ID NO: 59 - protein, 11 aa, Artificial Sequence
  Synthetic
QEWVQENYLEY

SEQ ID NO: 60 - protein, 11 aa, Artificial Sequence
  Synthetic
QDLVQEKYLEY

SEQ ID NO: 61 - protein, 11 aa, Artificial Sequence
  Synthetic
KDLVQEKYLEY

SEQ ID NO: 62 - protein, 11 aa, Artificial Sequence
  Synthetic
KDLVKENYLEY

SEQ ID NO: 63 - protein, 11 aa, Artificial Sequence
  Synthetic
KDFVKEKYLEY

SEQ ID NO: 64 - protein, 11 aa, Artificial Sequence
  Synthetic
KVWVQEHYLEY

SEQ ID NO: 65 - protein, 16 aa, Artificial Sequence
  Synthetic
RKLITDDFVKQKYLEY

SEQ ID NO: 66 - protein, 16 aa, Artificial Sequence
  Synthetic
KKLITDEFVKQKYLDY

SEQ ID NO: 67 - protein, 16 aa, Artificial Sequence
  Synthetic
KKLITEVFVRQKYLEY

SEQ ID NO: 68 - protein, 16 aa, Artificial Sequence
  Synthetic
KKLITEDFVRQRYLEY

SEQ ID NO: 69 - protein, 11 aa, Artificial Sequence
  Synthetic
EEFVQMNYLKY

SEQ ID NO: 70 - protein, 16 aa, Artificial Sequence
  Synthetic
KKLLTQDLVQENYLEY

SEQ ID NO: 71 - protein, 16 aa, Artificial Sequence
  Synthetic
KKLLTQDLVQEKYLEY